European Patent Specification EP 3 807 413 B1, published May 21, 2025. Title: ADENO-ASSOCIATED VIRUS VECTOR DELIVERY OF MUSCLE SPECIFIC MICRO-DYSTROPHIN TO TREAT MUSCULAR DYSTROPHY. Applicant: RESEARCH INSTITUTE AT NATIONWIDE CHILDREN'S HOSPITAL. The sequence listing filed with the application follows.

SEQUENCE LISTING (9 sequences)

SEQ ID NO: 1 - DNA, 3579 bp, Homo sapiens
atgctgtggtgggaggaggtggaggattgttatgaaagggaggacgtgcagaagaagacttttaccaagtgggtgaacgctcagttcagcaaatttgggaagcagcacatcgagaatctgttttccgacctgcaggatgggagacggctgctggatctgctggaaggactgactggccagaagctgcccaaagagaaggggagcactagggtgcacgccctgaacaacgtgaacaaagctctgagagtgctgcagaacaacaacgtggatctggtgaatattggcagtactgatatcgtggacgggaaccacaaactgacactgggcctgatctggaacattattctgcactggcaggtgaaaaatgtgatgaagaacatcatggccgggctgcagcagaccaattccgagaagatcctgctgtcttgggtgcggcagagcacccgcaactatccccaggtgaacgtgattaacttcactacatcctggagcgacgggctggccctgaatgctctgattcacagccacaggcctgatctgttcgactggaatagcgtggtgtgccagcagtctgccacacagcgcctggaacatgccttcaatatcgctcggtaccagctggggatcgaaaaactgctggacccagaggatgtggacactacatacccagataaaaagtctattctgatgtacattactagcctgttccaggtgctgccacagcaggtgtctattgaagccattcaggaggtggaaatgctgccccgcccccccaaagtgactaaagaggagcattttcagctgcatcatcagatgcattacagccagcagattaccgtgagcctggctcagggatatgagcgcaccagtagtccaaaaccacggttcaagtcctacgcttatacccaggctgcctacgtgacaactagcgaccctactagatccccctttccatcccagcacctggaggccccagaggacaagagctttgggtccagcctgatggaaagcgaggtgaatctggatcggtaccagacagccctggaggaggtgctgagctggctgctgagtgctgaagacacactgcaggcccagggcgaaatttccaatgacgtggaagtggtgaaggatcagttccacacacacgagggctatatgatggacctgacagctcaccaggggcgcgtgggcaatatcctgcagctgggctctaaactgatcggcaccgggaaactgagtgaggacgaggaaacagaagtgcaggagcagatgaacctgctgaacagccgctgggagtgtctgagagtggctagtatggagaagcagtccaacctgcaccgggtgctgatggacctgcagaaccagaaactgaaagagctgaacgactggctgacaaagactgaggaacgcacaaggaagatggaggaggagccactgggacccgacctggaggatctgaagagacaggtgcagcagcataaggtgctgcaggaggatctggaacaggagcaggtgcgggtgaactccctgacacatatggtggtggtggtggacgaatctagtggagatcacgccaccgccgccctggaggaacagctgaaggtgctgggggaccggtgggccaacatttgccggtggaccgaggacaggtgggtgctgctgcaggacatcctgctgaaatggcagaggctgaccgaggagcagtgtctgtttagtgcttggctgagcgagaaagaggacgccgtgaacaagatccacacaaccggctttaaggatcagaacgaaatgctgtctagcctgcagaaactggctgtgctgaaggccgatctggagaaaaagaagcagagcatgggcaaactgtatagcctgaaacaggacctgctgagcaccctgaagaacaagagcgtgacccagaagacagaagcctggctggataactttgcccgctgctgggacaacctggtgcagaaactggagaaaagtacagctcagatctctcaggctgtgaccacaacccagcctagcctgacccagacaaccgtgatggaaaccgtgaccaccgtgacaacccgcgaacagatcctggtgaaacatgcccaggaagagctgccacctccacctccccagaagaagagaaccctggagcggctgcaggagctgcaggaagccactgacgaactggacctgaagctgaggcaggccgaagtgattaaggggtcttggcagcctgtgggcgatctgctgattgattccctgcaggaccacctggaaaaggtgaaggctctgagaggcgaaattgctccactgaaggagaacgtgagtcatgtgaacgatctggctagacagctgacaacactgggcatccagctgagcccatacaatctgagcacactggaggacctgaataccaggtggaagctgctgcaggtggctgtggaagaccgggtgcggcagctgcatgaggcccatcgcgacttcggaccagccagccagcactttctgagcacatccgtgcaggggccctgggagagggccatttctcccaacaaggtgccctactatattaatcacgagacccagaccacttgttgggaccatcccaagatgacagaactgtaccagtccctggccgatctgaacaacgtgaggtttagcgcttacagaaccgctatgaagctgagacggctgcagaaggccctgtgcctggatctgctgtccctgtccgccgcctgcgatgccctggatcagcataatctgaagcagaacgatcagccaatggatatcctgcagatcatcaactgcctgaccactatctacgacaggctggagcaggagcacaacaacctggtgaacgtgcctctgtgcgtggatatgtgcctgaactggctgctgaacgtgtatgacactgggcgcaccggccggatcagagtgctgagttttaaaactgggattatctccctgtgtaaggcccacctggaggacaagtacaggtacctgttcaagcaggtggctagtagcactggattttgtgaccagcgccgcctgggactgctgctgcatgatagtatccagattcctagacagctgggagaggtggctagtttcggaggatctaacatcgaacccagcgtgcgcagctgtttccagtttgccaataacaaacctgaaatcgaggctgctctgttcctggattggatgcgcctggaaccacagagcatggtgtggctgcctgtgctgcacagagtggctgccgccgaaactgccaagcaccaggctaaatgcaacatctgcaaggaatgtcccattatcggctttcgctacaggagtctgaaacattttaactacgatatttgccagagctgcttcttttccggaagagtggccaaaggacacaagatgcactaccctatggtggaatattgcaccccaactacatctggcgaagatgtgcgcgattttgccaaggtgctgaagaataagtttcggactaagaggtacttcgccaagcacccccgcatggggtatctgccagtgcagacagtgctggaaggagacaatatggagaccgatacaatgtga

SEQ ID NO: 2 - DNA, 810 bp, Artificial Sequence
  Synthetic Promoter
gtttaaacaagcttgcatgtctaagctagacccttcagattaaaaataactgaggtaagggcctgggtaggggaggtggtgtgagacgctcctgtctctcctctatctgcccatcggccctttggggaggaggaatgtgcccaaggactaaaaaaaggccatggagccagaggggcgagggcaacagacctttcatgggcaaaccttggggccctgctgtctagcatgccccactacgggtctaggctgcccatgtaaggaggcaaggcctggggacacccgagatgcctggttataattaacccagacatgtggctgcccccccccccccaacacctgctgcctctaaaaataaccctgtccctggtggatcccctgcatgcgaagatcttcgaacaaggctgtgggggactgagggcaggctgtaacaggcttgggggccagggcttatacgtgcctgggactcccaaagtattactgttccatgttcccggcgaagggccagctgtcccccgccagctagactcagcacttagtttaggaaccagtgagcaagtcagcccttggggcagcccatacaaggccatggggctgggcaagctgcacgcctgggtccggggtgggcacggtgcccgggcaacgagctgaaagctcatctgctctcaggggcccctccctggggacagcccctcctggctagtcacaccctgtaggctcctctatataacccaggggcacaggggctgccctcattctaccaccacctccacagcacagacagacactcaggagccagccagcggcgcgccc

SEQ ID NO: 3 - DNA, 8562 bp, Adeno-associated virus
gcccaatacgcaaaccgcctctccccgcgcgttggccgattcattaatgcagctgcgcgctcgctcgctcactgaggccgcccgggcaaagcccgggcgtcgggcgacctttggtcgcccggcctcagtgagcgagcgagcgcgcagagagggagtggccaactccatcactaggggttccttgtagttaatgattaacccgccatgctacttatctacgtagccatgctctagagtttaaacaagcttgcatgtctaagctagacccttcagattaaaaataactgaggtaagggcctgggtaggggaggtggtgtgagacgctcctgtctctcctctatctgcccatcggccctttggggaggaggaatgtgcccaaggactaaaaaaaggccatggagccagaggggcgagggcaacagacctttcatgggcaaaccttggggccctgctgtctagcatgccccactacgggtctaggctgcccatgtaaggaggcaaggcctggggacacccgagatgcctggttataattaacccagacatgtggctgcccccccccccccaacacctgctgcctctaaaaataaccctgtccctggtggatcccctgcatgcgaagatcttcgaacaaggctgtgggggactgagggcaggctgtaacaggcttgggggccagggcttatacgtgcctgggactcccaaagtattactgttccatgttcccggcgaagggccagctgtcccccgccagctagactcagcacttagtttaggaaccagtgagcaagtcagcccttggggcagcccatacaaggccatggggctgggcaagctgcacgcctgggtccggggtgggcacggtgcccgggcaacgagctgaaagctcatctgctctcaggggcccctccctggggacagcccctcctggctagtcacaccctgtaggctcctctatataacccaggggcacaggggctgccctcattctaccaccacctccacagcacagacagacactcaggagcagccagcggcgcgcccaggtaagtttagtctttttgtcttttatttcaggtcccggatccggtggtggtgcaaatcaaagaactgctcctcagtggatgttgcctttacttctaggcctgtacggaagtgttacttctgctctaaaagctgcggaattgtacccgcggccgccaccatgctgtggtgggaggaggtggaggattgttatgaaagggaggacgtgcagaagaagacttttaccaagtgggtgaacgctcagttcagcaaatttgggaagcagcacatcgagaatctgttttccgacctgcaggatgggagacggctgctggatctgctggaaggactgactggccagaagctgcccaaagagaaggggagcactagggtgcacgccctgaacaacgtgaacaaagctctgagagtgctgcagaacaacaacgtggatctggtgaatattggcagtactgatatcgtggacgggaaccacaaactgacactgggcctgatctggaacattattctgcactggcaggtgaaaaatgtgatgaagaacatcatggccgggctgcagcagaccaattccgagaagatcctgctgtcttgggtgcggcagagcacccgcaactatccccaggtgaacgtgattaacttcactacatcctggagcgacgggctggccctgaatgctctgattcacagccacaggcctgatctgttcgactggaatagcgtggtgtgccagcagtctgccacacagcgcctggaacatgccttcaatatcgctcggtaccagctggggatcgaaaaactgctggacccagaggatgtggacactacatacccagataaaaagtctattctgatgtacattactagcctgttccaggtgctgccacagcaggtgtctattgaagccattcaggaggtggaaatgctgccccgcccccccaaagtgactaaagaggagcattttcagctgcatcatcagatgcattacagccagcagattaccgtgagcctggctcagggatatgagcgcaccagtagtccaaaaccacggttcaagtcctacgcttatacccaggctgcctacgtgacaactagcgaccctactagatccccctttccatcccagcacctggaggccccagaggacaagagctttgggtccagcctgatggaaagcgaggtgaatctggatcggtaccagacagccctggaggaggtgctgagctggctgctgagtgctgaagacacactgcaggcccagggcgaaatttccaatgacgtggaagtggtgaaggatcagttccacacacacgagggctatatgatggacctgacagctcaccaggggcgcgtgggcaatatcctgcagctgggctctaaactgatcggcaccgggaaactgagtgaggacgaggaaacagaagtgcaggagcagatgaacctgctgaacagccgctgggagtgtctgagagtggctagtatggagaagcagtccaacctgcaccgggtgctgatggacctgcagaaccagaaactgaaagagctgaacgactggctgacaaagactgaggaacgcacaaggaagatggaggaggagccactgggacccgacctggaggatctgaagagacaggtgcagcagcataaggtgctgcaggaggatctggaacaggagcaggtgcgggtgaactccctgacacatatggtggtggtggtggacgaatctagtggagatcacgccaccgccgccctggaggaacagctgaaggtgctgggggaccggtgggccaacatttgccggtggaccgaggacaggtgggtgctgctgcaggacatcctgctgaaatggcagaggctgaccgaggagcagtgtctgtttagtgcttggctgagcgagaaagaggacgccgtgaacaagatccacacaaccggctttaaggatcagaacgaaatgctgtctagcctgcagaaactggctgtgctgaaggccgatctggagaaaaagaagcagagcatgggcaaactgtatagcctgaaacaggacctgctgagcaccctgaagaacaagagcgtgacccagaagacagaagcctggctggataactttgcccgctgctgggacaacctggtgcagaaactggagaaaagtacagctcagatctctcaggctgtgaccacaacccagcctagcctgacccagacaaccgtgatggaaaccgtgaccaccgtgacaacccgcgaacagatcctggtgaaacatgcccaggaagagctgccacctccacctccccagaagaagagaaccctggagcggctgcaggagctgcaggaagccactgacgaactggacctgaagctgaggcaggccgaagtgattaaggggtcttggcagcctgtgggcgatctgctgattgattccctgcaggaccacctggaaaaggtgaaggctctgagaggcgaaattgctccactgaaggagaacgtgagtcatgtgaacgatctggctagacagctgacaacactgggcatccagctgagcccatacaatctgagcacactggaggacctgaataccaggtggaagctgctgcaggtggctgtggaagaccgggtgcggcagctgcatgaggcccatcgcgacttcggaccagccagccagcactttctgagcacatccgtgcaggggccctgggagagggccatttctcccaacaaggtgccctactatattaatcacgagacccagaccacttgttgggaccatcccaagatgacagaactgtaccagtccctggccgatctgaacaacgtgaggtttagcgcttacagaaccgctatgaagctgagacggctgcagaaggccctgtgcctggatctgctgtccctgtccgccgcctgcgatgccctggatcagcataatctgaagcagaacgatcagccaatggatatcctgcagatcatcaactgcctgaccactatctacgacaggctggagcaggagcacaacaacctggtgaacgtgcctctgtgcgtggatatgtgcctgaactggctgctgaacgtgtatgacactgggcgcaccggccggatcagagtgctgagttttaaaactgggattatctccctgtgtaaggcccacctggaggacaagtacaggtacctgttcaagcaggtggctagtagcactggattttgtgaccagcgccgcctgggactgctgctgcatgatagtatccagattcctagacagctgggagaggtggctagtttcggaggatctaacatcgaacccagcgtgcgcagctgtttccagtttgccaataacaaacctgaaatcgaggctgctctgttcctggattggatgcgcctggaaccacagagcatggtgtggctgcctgtgctgcacagagtggctgccgccgaaactgccaagcaccaggctaaatgcaacatctgcaaggaatgtcccattatcggctttcgctacaggagtctgaaacattttaactacgatatttgccagagctgcttcttttccggaagagtggccaaaggacacaagatgcactaccctatggtggaatattgcaccccaactacatctggcgaagatgtgcgcgattttgccaaggtgctgaagaataagtttcggactaagaggtacttcgccaagcacccccgcatggggtatctgccagtgcagacagtgctggaaggagacaatatggagaccgatacaatgtgagcggccgcaataaaagatctttattttcattagatctgtgtgttggttttttgtgtgtctagagcatggctacgtagataagtagcatggcgggttaatcattaactacaaggaacccctagtgatggagttggccactccctctctgcgcgctcgctcgctcactgaggccgggcgaccaaaggtcgcccgacgcccgggctttgcccgggcggcctcagtgagcgagcgagcgcgcagctggcgtaatagcgaagaggcccgcaccgatcgcccttcccaacagttgcgcagcctgaatggcgaatggcgattccgttgcaatggctggcggtaatattgttctggatattaccagcaaggccgatagtttgagttcttctactcaggcaagtgatgttattactaatcaaagaagtattgcgacaacggttaatttgcgtgatggacagactcttttactcggtggcctcactgattataaaaacacttctcaggattctggcgtaccgttcctgtctaaaatccctttaatcggcctcctgtttagctcccgctctgattctaacgaggaaagcacgttatacgtgctcgtcaaagcaaccatagtacgcgccctgtagcggcgcattaagcgcggcgggtgtggtggttacgcgcagcgtgaccgctacacttgccagcgccctagcgcccgctcctttcgctttcttcccttcctttctcgccacgttcgccggctttccccgtcaagctctaaatcgggggctccctttagggttccgatttagtgctttacggcacctcgaccccaaaaaacttgattagggtgatggttcacgtagtgggccatcgccctgatagacggtttttcgccctttgacgttggagtccacgttctttaatagtggactcttgttccaaactggaacaacactcaaccctatctcggtctattcttttgatttataagggattttgccgatttcggcctattggttaaaaaatgagctgatttaacaaaaatttaacgcgaattttaacaaaatattaacgcttacaatttaaatatttgcttatacaatcttcctgtttttggggcttttctgattatcaaccggggtacatatgattgacatgctagttttacgattaccgttcatcgattctcttgtttgctccagactctcaggcaatgacctgatagcctttgtagagacctctcaaaaatagctaccctctccggcatgaatttatcagctagaacggttgaatatcatattgatggtgatttgactgtctccggcctttctcacccgtttgaatctttacctacacattactcaggcattgcatttaaaatatatgagggttctaaaaatttttatccttgcgttgaaataaaggcttctcccgcaaaagtattacagggtcataatgtttttggtacaaccgatttagctttatgctctgaggctttattgcttaattttgctaattctttgccttgcctgtatgatttattggatgttggaatcgcctgatgcggtattttctccttacgcatctgtgcggtatttcacaccgcatatggtgcactctcagtacaatctgctctgatgccgcatagttaagccagccccgacacccgccaacacccgctgacgcgccctgacgggcttgtctgctcccggcatccgcttacagacaagctgtgaccgtctccgggagctgcatgtgtcagaggttttcaccgtcatcaccgaaacgcgcgagacgaaagggcctcgtgatacgcctatttttataggttaatgtcatgataataatggtttcttagacgtcaggtggcacttttcggggaaatgtgcgcggaacccctatttgtttatttttctaaatacattcaaatatgtatccgctcatgagacaataaccctgataaatgcttcaataatattgaaaaaggaagagtatgagtattcaacatttccgtgtcgcccttattcccttttttgcggcattttgccttcctgtttttgctcacccagaaacgctggtgaaagtaaaagatgctgaagatcagttgggtgcacgagtgggttacatcgaactggatctcaacagcggtaagatccttgagagttttcgccccgaagaacgttttccaatgatgagcacttttaaagttctgctatgtggcgcggtattatcccgtattgacgccgggcaagagcaactcggtcgccgcatacactattctcagaatgacttggttgagtactcaccagtcacagaaaagcatcttacggatggcatgacagtaagagaattatgcagtgctgccataaccatgagtgataacactgcggccaacttacttctgacaacgatcggaggaccgaaggagctaaccgcttttttgcacaacatgggggatcatgtaactcgccttgatcgttgggaaccggagctgaatgaagccataccaaacgacgagcgtgacaccacgatgcctgtagcaatggcaacaacgttgcgcaaactattaactggcgaactacttactctagcttcccggcaacaattaatagactggatggaggcggataaagttgcaggaccacttctgcgctcggcccttccggctggctggtttattgctgataaatctggagccggtgagcgtgggtctcgcggtatcattgcagcactggggccagatggtaagccctcccgtatcgtagttatctacacgacggggagtcaggcaactatggatgaacgaaatagacagatcgctgagataggtgcctcactgattaagcattggtaactgtcagaccaagtttactcatatatactttagattgatttaaaacttcatttttaatttaaaaggatctaggtgaagatcctttttgataatctcatgaccaaaatcccttaacgtgagttttcgttccactgagcgtcagaccccgtagaaaagatcaaaggatcttcttgagatcctttttttctgcgcgtaatctgctgcttgcaaacaaaaaaaccaccgctaccagcggtggtttgtttgccggatcaagagctaccaactctttttccgaaggtaactggcttcagcagagcgcagataccaaatactgttcttctagtgtagccgtagttaggccaccacttcaagaactctgtagcaccgcctacatacctcgctctgctaatcctgttaccagtggctgctgccagtggcgataagtcgtgtcttaccgggttggactcaagacgatagttaccggataaggcgcagcggtcgggctgaacggggggttcgtgcacacagcccagcttggagcgaacgacctacaccgaactgagatacctacagcgtgagctatgagaaagcgccacgcttcccgaagggagaaaggcggacaggtatccggtaagcggcagggtcggaacaggagagcgcacgagggagcttccagggggaaacgcctggtatctttatagtcctgtcgggtttcgccacctctgacttgagcgtcgatttttgtgatgctcgtcaggggggcggagcctatggaaaaacgccagcaacgcggcctttttacggttcctggccttttgctggccttttgctcacatgttctttcctgcgttatcccctgattctgtggataaccgtattaccgcctttgagtgagctgataccgctcgccgcagccgaacgaccgagcgcagcgagtcagtgagcgaggaagcggaagagc

SEQ ID NO: 4 - DNA, 564 bp, Artificial Sequence
  Synthetic Promoter
cagccactatgggtctaggctgcccatgtaaggaggcaaggcctggggacacccgagatgcctggttataattaacccagacatgtggctgctccccccccccaacacctgctgcctgagcctcacccccaccccggtgcctgggtcttaggctctgtacaccatggaggagaagctcgctctaaaaataaccctgtccctggtgggctgtgggggactgagggcaggctgtaacaggcttgggggccagggcttatacgtgcctgggactcccaaagtattactgttccatgttcccggcgaagggccagctgtcccccgccagctagactcagcacttagtttaggaaccagtgagcaagtcagcccttggggcagcccatacaaggccatggggctgggcaagctgcacgcctgggtccggggtgggcacggtgcccgggcaacgagctgaaagctcatctgctctcaggggcccctccctggggacagcccctcctggctagtcacaccctgtaggctcctctatataacccaggggcacaggggctgcccccgggtcac

SEQ ID NO: 5 - DNA, 8409 bp, Adeno-associated virus
gcccaatacgcaaaccgcctctccccgcgcgttggccgattcattaatgcagctggcgcgctcgctcgctcactgaggccgcccgggcaaagcccgggcgtcgggcgacctttggtcgcccggcctcagtgagcgagcgagcgcgcagagagggagtggccaactccatcactaggggttccttgtagttaatgattaacccgccatgctaattatctacgtagccatgtctagacagccactatgggtctaggctgcccatgtaaggaggcaaggcctggggacacccgagatgcctggttataattaacccagacatgtggctgctccccccccccaacacctgctgcctgagcctcacccccaccccggtgcctgggtcttaggctctgtacaccatggaggagaagctcgctctaaaaataaccctgtccctggtgggctgtgggggactgagggcaggctgtaacaggcttgggggccagggcttatacgtgcctgggactcccaaagtattactgttccatgttcccggcgaagggccagctgtcccccgccagctagactcagcacttagtttaggaaccagtgagcaagtcagcccttggggcagcccatacaaggccatggggctgggcaagctgcacgcctgggtccggggtgggcacggtgcccgggcaacgagctgaaagctcatctgctctcaggggcccctccctggggacagcccctcctggctagtcacaccctgtaggctcctctatataacccaggggcacaggggctgcccccgggtcaccaccacctccacagcacagacagacactcaggagccagccagccaggtaagtttagtctttttgtcttttatttcaggtcccggatccggtggtggtgcaaatcaaagaactgctcctcagtggatgttgcctttacttctaggcctgtacggaagtgttacttctgctctaaaagctgcggaattgtacccgcggccgccaccatgctgtggtgggaggaggtggaggattgttatgaaagggaggacgtgcagaagaagacttttaccaagtgggtgaacgctcagttcagcaaatttgggaagcagcacatcgagaatctgttttccgacctgcaggatgggagacggctgctggatctgctggaaggactgactggccagaagctgcccaaagagaaggggagcactagggtgcacgccctgaacaacgtgaacaaagctctgagagtgctgcagaacaacaacgtggatctggtgaatattggcagtactgatatcgtggacgggaaccacaaactgacactgggcctgatctggaacattattctgcactggcaggtgaaaaatgtgatgaagaacatcatggccgggctgcagcagaccaattccgagaagatcctgctgtcttgggtgcggcagagcacccgcaactatccccaggtgaacgtgattaacttcactacatcctggagcgacgggctggccctgaatgctctgattcacagccacaggcctgatctgttcgactggaatagcgtggtgtgccagcagtctgccacacagcgcctggaacatgccttcaatatcgctcggtaccagctggggatcgaaaaactgctggacccagaggatgtggacactacatacccagataaaaagtctattctgatgtacattactagcctgttccaggtgctgccacagcaggtgtctattgaagccattcaggaggtggaaatgctgccccgcccccccaaagtgactaaagaggagcattttcagctgcatcatcagatgcattacagccagcagattaccgtgagcctggctcagggatatgagcgcaccagtagtccaaaaccacggttcaagtcctacgcttatacccaggctgcctacgtgacaactagcgaccctactagatccccctttccatcccagcacctggaggccccagaggacaagagctttgggtccagcctgatggaaagcgaggtgaatctggatcggtaccagacagccctggaggaggtgctgagctggctgctgagtgctgaagacacactgcaggcccagggcgaaatttccaatgacgtggaagtggtgaaggatcagttccacacacacgagggctatatgatggacctgacagctcaccaggggcgcgtgggcaatatcctgcagctgggctctaaactgatcggcaccgggaaactgagtgaggacgaggaaacagaagtgcaggagcagatgaacctgctgaacagccgctgggagtgtctgagagtggctagtatggagaagcagtccaacctgcaccgggtgctgatggacctgcagaaccagaaactgaaagagctgaacgactggctgacaaagactgaggaacgcacaaggaagatggaggaggagccactgggacccgacctggaggatctgaagagacaggtgcagcagcataaggtgctgcaggaggatctggaacaggagcaggtgcgggtgaactccctgacacatatggtggtggtggtggacgaatctagtggagatcacgccaccgccgccctggaggaacagctgaaggtgctgggggaccggtgggccaacatttgccggtggaccgaggacaggtgggtgctgctgcaggacatcctgctgaaatggcagaggctgaccgaggagcagtgtctgtttagtgcttggctgagcgagaaagaggacgccgtgaacaagatccacacaaccggctttaaggatcagaacgaaatgctgtctagcctgcagaaactggctgtgctgaaggccgatctggagaaaaagaagcagagcatgggcaaactgtatagcctgaaacaggacctgctgagcaccctgaagaacaagagcgtgacccagaagacagaagcctggctggataactttgcccgctgctgggacaacctggtgcagaaactggagaaaagtacagctcagatctctcaggctgtgaccacaacccagcctagcctgacccagacaaccgtgatggaaaccgtgaccaccgtgacaacccgcgaacagatcctggtgaaacatgcccaggaagagctgccacctccacctccccagaagaagagaaccctggagcggctgcaggagctgcaggaagccactgacgaactggacctgaagctgaggcaggccgaagtgattaaggggtcttggcagcctgtgggcgatctgctgattgattccctgcaggaccacctggaaaaggtgaaggctctgagaggcgaaattgctccactgaaggagaacgtgagtcatgtgaacgatctggctagacagctgacaacactgggcatccagctgagcccatacaatctgagcacactggaggacctgaataccaggtggaagctgctgcaggtggctgtggaagaccgggtgcggcagctgcatgaggcccatcgcgacttcggaccagccagccagcactttctgagcacatccgtgcaggggccctgggagagggccatttctcccaacaaggtgccctactatattaatcacgagacccagaccacttgttgggaccatcccaagatgacagaactgtaccagtccctggccgatctgaacaacgtgaggtttagcgcttacagaaccgctatgaagctgagacggctgcagaaggccctgtgcctggatctgctgtccctgtccgccgcctgcgatgccctggatcagcataatctgaagcagaacgatcagccaatggatatcctgcagatcatcaactgcctgaccactatctacgacaggctggagcaggagcacaacaacctggtgaacgtgcctctgtgcgtggatatgtgcctgaactggctgctgaacgtgtatgacactgggcgcaccggccggatcagagtgctgagttttaaaactgggattatctccctgtgtaaggcccacctggaggacaagtacaggtacctgttcaagcaggtggctagtagcactggattttgtgaccagcgccgcctgggactgctgctgcatgatagtatccagattcctagacagctgggagaggtggctagtttcggaggatctaacatcgaacccagcgtgcgcagctgtttccagtttgccaataacaaacctgaaatcgaggctgctctgttcctggattggatgcgcctggaaccacagagcatggtgtggctgcctgtgctgcacagagtggctgccgccgaaactgccaagcaccaggctaaatgcaacatctgcaaggaatgtcccattatcggctttcgctacaggagtctgaaacattttaactacgatatttgccagagctgcttcttttccggaagagtggccaaaggacacaagatgcactaccctatggtggaatattgcaccccaactacatctggcgaagatgtgcgcgattttgccaaggtgctgaagaataagtttcggactaagaggtacttcgccaagcacccccgcatggggtatctgccagtgcagacagtgctggaaggagacaatatggagaccgatacaatgtgagcggccgcaataaaagatctttattttcattagatctgtgtgttggttttttgtgtgtctagagcatggctacgtagataagtagcatggcgggttaatcattaactacaaggaacccctagtgatggagttggccactccctctctgcgcgctcgctcgctcactgaggccgggcgaccaaaggtcgcccgacgcccgggctttgcccgggcggcctcagtgagcgagcgagcgcgccagctggcgtaatagcgaagaggcccgcaccgatcgcccttcccaacagttgcgcagcctgaatggcgaatggaagttccagacgattgagcgtcaaaatgtaggtatttccatgagcgtttttcctgttgcaatggctggcggtaatattgttctggatattaccagcaaggccgatagtttgagttcttctactcaggcaagtgatgttattactaatcaaagaagtattgcgacaacggttaatttgcgtgatggacagactcttttactcggtggcctcactgattataaaaacacttctcaggattctggcgtaccgttcctgtctaaaatccctttaatcggcctcctgtttagctcccgctctgattctaacgaggaaagcacgttatacgtgctcgtcaaagcaaccatagtacgcgccctgtagcggcgcattaagcgcggcgggtgtggtggttacgcgcagcgtgaccgctacacttgccagcgccctagcgcccgctcctttcgctttcttcccttcctttctcgccacgttcgccggctttccccgtcaagctctaaatcgggggctccctttagggttccgatttagtgatttacggcacctcgaccccaaaaaacttgattagggtgatggttcacgtagtgggccatcgccctgatagacggtttttcgccctttgacgttggagtccacgttctttaatagtggactcttgttccaaactggaacaacactcaaccctatctcggtctattcttttgatttataagggattttgccgatttcggcctattggttaaaaaatgagctgatttaacaaaaatttaacgcgaattttaacaaaatattaacgtttacaatttaaatatttgcttatacaatcttcctgtttttggggcttttctgattatcaaccggggtacatatgattgacatgctagttttacgattaccgttcatcgattctcttgtttgctccagactctcaggcaatgacctgatagcctttgtagagacctctcaaaaatagctaccctctccggcatgaatttatcagctagaacggttgaatatcatattgatggtgatttgactgtctccggcctttctcacccgtttgaatctttacctacacattactcaggcattgcatttaaaatatatgagggttctaaaaatttttatccttgcgttgaaataaaggcttctcccgcaaaagtattacagggtcataatgtttttggtacaaccgatttagctttatgctctgaggctttattgcttaattttgctaattctttgccttgcctgtatgatttattggatgttggaagttcctgatgcggtattttctccttacgcatctgtgcggtatttcacaccgcatatggtgcactctcagtacaatctgctctgatgccgcatagttaagccagccccgacacccgccaacacccgctgacgcgccctgacgggcttgtctgctcccggcatccgcttacagacaagctgtgaccgtctccgggagctgcatgtgtcagaggttttcaccgtcatcaccgaaacgcgcgagacgaaagggcctcgtgatacgcctatttttataggttaatgtcatgataataatggtttcttagacgtcaggtggcacttttcggggaaatgtgcgcggaacccctatttgtttatttttctaaatacattcaaatatgtatccgctcatgagacaataaccctgataaatgcttcaataatattgaaaaaggaagagtatgagtattcaacatttccgtgtcgcccttattcccttttttgcggcattttgccttcctgtttttgctcacccagaaacgctggtgaaagtaaaagatgctgaagatcagttgggtgcacgagtgggttacatcgaactggatctcaacagcggtaagatccttgagagttttcgccccgaagaacgttttccaatgatgagcacttttaaagttctgctatgtggcgcggtattatcccgtattgacgccgggcaagagcaactcggtcgccgcatacactattctcagaatgacttggttgagtactcaccagtcacagaaaagcatcttacggatggcatgacagtaagagaattatgcagtgctgccataaccatgagtgataacactgcggccaacttacttctgacaacgatcggaggaccgaaggagctaaccgcttttttgcacaacatgggggatcatgtaactcgccttgatcgttgggaaccggagctgaatgaagccataccaaacgacgagcgtgacaccacgatgcctgtagcaatggcaacaacgttgcgcaaactattaactggcgaactacttactctagcttcccggcaacaattaatagactggatggaggcggataaagttgcaggaccacttctgcgctcggcccttccggctggctggtttattgctgataaatctggagccggtgagcgtgggtctcgcggtatcattgcagcactggggccagatggtaagccctcccgtatcgtagttatctacacgacggggagtcaggcaactatggatgaacgaaatagacagatcgctgagataggtgcctcactgattaagcattggtaactgtcagaccaagtttactcatatatactttagattgatttaaaacttcatttttaatttaaaaggatctaggtgaagatcctttttgataatctcatgaccaaaatcccttaacgtgagttttcgttccactgagcgtcagaccccgtagaaaagatcaaaggatcttcttgagatcctttttttctgcgcgtaatctgctgcttgcaaacaaaaaaaccaccgctaccagcggtggtttgtttgccggatcaagagctaccaactctttttccgaaggtaactggcttcagcagagcgcagataccaaatactgtccttctagtgtagccgtagttaggccaccacttcaagaactctgtagcaccgcgtacatacctcgctctgctaatcctgttaccagtggctgctgccagtggcgataagtcgtgtcttaccgggttggactcaagacgatagttaccggataaggcgcagcggtcgggctgaacggggggttcgtgcacacagcccagcttggagcgaacgacctacaccgaactgagatacctacagcgtgagctatgagaaagcgccacgcttcccgaagggagaaaggcggacaggtatccggtaagcggcagggtcggaacaggagagcgcacgagggagcttccagggggaaacgcctggtatctttatagtcctgtcgggtttcgccacctctgacttgagcgtcgatttttgtgatgctcgtcaggggggcggagcctatggaaaaacgccagcaacgcggcctttttacggttcctggccttttgctggccttttgctcacatgttctttcctgcgttatcccctgattctgtggataaccgtattaccgggtttgagtgagctgataccgctcgccgcagccgaacgaccgagcgcagcgagtcagtgagcgaccaagcggaagagc

SEQ ID NO: 6 - DNA, 8611 bp, Adeno-associated virus
gcccaatacgcaaaccgcctctccccgcgcgttggccgattcattaatgcagctggcgcgctcgctcgctcactgaggccgcccgggcaaagcccgggcgtcgggcgacctttggtcgcccggcctcagtgagcgagcgagcgcgcagagagggagtggccaactccatcactaggggttccttgtagttaatgattaacccgccatgctaattatctacgtagccatgtctagagtttaaacaagcttgcatgtctaagctagacccttcagattaaaaataactgaggtaagggcctgggtaggggaggtggtgtgagacgctcctgtctctcctctatctgcccatcggccctttggggaggaggaatgtgcccaaggactaaaaaaaggccatggagccagaggggcgagggcaacagacctttcatgggcaaaccttggggccctgctgtctagcatgccccactacgggtctaggctgcccatgtaaggaggcaaggcctggggacacccgagatgcctggttataattaacccagacatgtggctgcccccccccccccaacacctgctgcctctaaaaataaccctgtccctggtggatcccctgcatgcgaagatcttcgaacaaggctgtgggggactgagggcaggctgtaacaggcttgggggccagggcttatacgtgcctgggactcccaaagtattactgttccatgttcccggcgaagggccagctgtcccccgccagctagactcagcacttagtttaggaaccagtgagcaagtcagcccttggggcagcccatacaaggccatggggctgggcaagctgcacgcctgggtccggggtgggcacggtgcccgggcaacgagctgaaagctcatctgctctcaggggcccctccctggggacagcccctcctggctagtcacaccctgtaggctcctctatataacccaggggcacaggggctgccctcattctaccaccacctccacagcacagacagacactcaggagccagccagcggcgcgcccaggtaagtttagtctttttgtcttttatttcaggtcccggatccggtggtggtgcaaatcaaagaactgctcctcagtggatgttgcctttacttctaggcctgtacggaagtgttacttctgctctaaaagctgcggaattgtacccgcggccgccaccatgctgtggtgggaggaggtggaggattgttatgaaagggaggacgtgcagaagaagacttttaccaagtgggtgaacgctcagttcagcaaatttgggaagcagcacatcgagaatctgttttccgacctgcaggatgggagacggctgctggatctgctggaaggactgactggccagaagctgcccaaagagaaggggagcactagggtgcacgccctgaacaacgtgaacaaagctctgagagtgctgcagaacaacaacgtggatctggtgaatattggcagtactgatatcgtggacgggaaccacaaactgacactgggcctgatctggaacattattctgcactggcaggtgaaaaatgtgatgaagaacatcatggccgggctgcagcagaccaattccgagaagatcctgctgtcttgggtgcggcagagcacccgcaactatccccaggtgaacgtgattaacttcactacatcctggagcgacgggctggccctgaatgctctgattcacagccacaggcctgatctgttcgactggaatagcgtggtgtgccagcagtctgccacacagcgcctggaacatgccttcaatatcgctcggtaccagctggggatcgaaaaactgctggacccagaggatgtggacactacatacccagataaaaagtctattctgatgtacattactagcctgttccaggtgctgccacagcaggtgtctattgaagccattcaggaggtggaaatgctgccccgcccccccaaagtgactaaagaggagcattttcagctgcatcatcagatgcattacagccagcagattaccgtgagcctggctcagggatatgagcgcaccagtagtccaaaaccacggttcaagtcctacgcttatacccaggctgcctacgtgacaactagcgaccctactagatccccctttccatcccagcacctggaggccccagaggacaagagctttgggtccagcctgatggaaagcgaggtgaatctggatcggtaccagacagccctggaggaggtgctgagctggctgctgagtgctgaagacacactgcaggcccagggcgaaatttccaatgacgtggaagtggtgaaggatcagttccacacacacgagggctatatgatggacctgacagctcaccaggggcgcgtgggcaatatcctgcagctgggctctaaactgatcggcaccgggaaactgagtgaggacgaggaaacagaagtgcaggagcagatgaacctgctgaacagccgctgggagtgtctgagagtggctagtatggagaagcagtccaacctgcaccgggtgctgatggacctgcagaaccagaaactgaaagagctgaacgactggctgacaaagactgaggaacgcacaaggaagatggaggaggagccactgggacccgacctggaggatctgaagagacaggtgcagcagcataaggtgctgcaggaggatctggaacaggagcaggtgcgggtgaactccctgacacatatggtggtggtggtggacgaatctagtggagatcacgccaccgccgccctggaggaacagctgaaggtgctgggggaccggtgggccaacatttgccggtggaccgaggacaggtgggtgctgctgcaggacatcctgctgaaatggcagaggctgaccgaggagcagtgtctgtttagtgcttggctgagcgagaaagaggacgccgtgaacaagatccacacaaccggctttaaggatcagaacgaaatgctgtctagcctgcagaaactggctgtgctgaaggccgatctggagaaaaagaagcagagcatgggcaaactgtatagcctgaaacaggacctgctgagcaccctgaagaacaagagcgtgacccagaagacagaagcctggctggataactttgcccgctgctgggacaacctggtgcagaaactggagaaaagtacagctcagatctctcaggctgtgaccacaacccagcctagcctgacccagacaaccgtgatggaaaccgtgaccaccgtgacaacccgcgaacagatcctggtgaaacatgcccaggaagagctgccacctccacctccccagaagaagagaaccctggagcggctgcaggagctgcaggaagccactgacgaactggacctgaagctgaggcaggccgaagtgattaaggggtcttggcagcctgtgggcgatctgctgattgattccctgcaggaccacctggaaaaggtgaaggctctgagaggcgaaattgctccactgaaggagaacgtgagtcatgtgaacgatctggctagacagctgacaacactgggcatccagctgagcccatacaatctgagcacactggaggacctgaataccaggtggaagctgctgcaggtggctgtggaagaccgggtgcggcagctgcatgaggcccatcgcgacttcggaccagccagccagcactttctgagcacatccgtgcaggggccctgggagagggccatttctcccaacaaggtgccctactatattaatcacgagacccagaccacttgttgggaccatcccaagatgacagaactgtaccagtccctggccgatctgaacaacgtgaggtttagcgcttacagaaccgctatgaagctgagacggctgcagaaggccctgtgcctggatctgctgtccctgtccgccgcctgcgatgccctggatcagcataatctgaagcagaacgatcagccaatggatatcctgcagatcatcaactgcctgaccactatctacgacaggctggagcaggagcacaacaacctggtgaacgtgcctctgtgcgtggatatgtgcctgaactggctgctgaacgtgtatgacactgggcgcaccggccggatcagagtgctgagttttaaaactgggattatctccctgtgtaaggcccacctggaggacaagtacaggtacctgttcaagcaggtggctagtagcactggattttgtgaccagcgccgcctgggactgctgctgcatgatagtatccagattcctagacagctgggagaggtggctagtttcggaggatctaacatcgaacccagcgtgcgcagctgtttccagtttgccaataacaaacctgaaatcgaggctgctctgttcctggattggatgcgcctggaaccacagagcatggtgtggctgcctgtgctgcacagagtggctgccgccgaaactgccaagcaccaggctaaatgcaacatctgcaaggaatgtcccattatcggctttcgctacaggagtctgaaacattttaactacgatatttgccagagctgcttcttttccggaagagtggccaaaggacacaagatgcactaccctatggtggaatattgcaccccaactacatctggcgaagatgtgcgcgattttgccaaggtgctgaagaataagtttcggactaagaggtacttcgccaagcacccccgcatggggtatctgccagtgcagacagtgctggaaggagacaatatggagaccgatacaatgtgagcggccgcaataaaagatctttattttcattagatctgtgtgttggttttttgtgtgtctagagcatggctacgtagataagtagcatggcgggttaatcattaactacaaggaacccctagtgatggagttggccactccctctctgcgcgctcgctcgctcactgaggccgggcgaccaaaggtcgcccgacgcccgggctttgcccgggcggcctcagtgagcgagcgagcgcgccagctggcgtaatagcgaagaggcccgcaccgatcgcccttcccaacagttgcgcagcctgaatggcgaatggaagttccagacgattgagcgtcaaaatgtaggtatttccatgagcgtttttcctgttgcaatggctggcggtaatattgttctggatattaccagcaaggccgatagtttgagttcttctactcaggcaagtgatgttattactaatcaaagaagtattgcgacaacggttaatttgcgtgatggacagactcttttactcggtggcctcactgattataaaaacacttctcaggattctggcgtaccgttcctgtctaaaatccctttaatcggcctcctgtttagctcccgctctgattctaacgaggaaagcacgttatacgtgctcgtcaaagcaaccatagtacgcgccctgtagcggcgcattaagcgcggcgggtgtggtggttacgcgcagcgtgaccgctacacttgccagcgccctagcgcccgctcctttcgctttcttcccttcctttctcgccacgttcgccggctttccccgtcaagctctaaatcgggggctccctttagggttccgatttagtgatttacggcacctcgaccccaaaaaacttgattagggtgatggttcacgtagtgggccatcgccctgatagacggtttttcgccctttgacgttggagtccacgttctttaatagtggactcttgttccaaactggaacaacactcaaccctatctcggtctattcttttgatttataagggattttgccgatttcggcctattggttaaaaaatgagctgatttaacaaaaatttaacgcgaattttaacaaaatattaacgtttacaatttaaatatttgcttatacaatcttcctgtttttggggcttttctgattatcaaccggggtacatatgattgacatgctagttttacgattaccgttcatcgattctcttgtttgctccagactctcaggcaatgacctgatagcctttgtagagacctctcaaaaatagctaccctctccggcatgaatttatcagctagaacggttgaatatcatattgatggtgatttgactgtctccggcctttctcacccgtttgaatctttacctacacattactcaggcattgcatttaaaatatatgagggttctaaaaatttttatccttgcgttgaaataaaggcttctcccgcaaaagtattacagggtcataatgtttttggtacaaccgatttagctttatgctctgaggctttattgcttaattttgctaattctttgccttgcctgtatgatttattggatgttggaagttcctgatgcggtattttctccttacgcatctgtgcggtatttcacaccgcatatggtgcactctcagtacaatctgctctgatgccgcatagttaagccagccccgacacccgccaacacccgctgacgcgccctgacgggcttgtctgctcccggcatccgcttacagacaagctgtgaccgtctccgggagctgcatgtgtcagaggttttcaccgtcatcaccgaaacgcgcgagacgaaagggcctcgtgatacgcctatttttataggttaatgtcatgataataatggtttcttagacgtcaggtggcacttttcggggaaatgtgcgcggaacccctatttgtttatttttctaaatacattcaaatatgtatccgctcatgagacaataaccctgataaatgcttcaataatattgaaaaaggaagagtatgagtattcaacatttccgtgtcgcccttattcccttttttgcggcattttgccttcctgtttttgctcacccagaaacgctggtgaaagtaaaagatgctgaagatcagttgggtgcacgagtgggttacatcgaactggatctcaacagcggtaagatccttgagagttttcgccccgaagaacgttttccaatgatgagcacttttaaagttctgctatgtggcgcggtattatcccgtattgacgccgggcaagagcaactcggtcgccgcatacactattctcagaatgacttggttgagtactcaccagtcacagaaaagcatcttacggatggcatgacagtaagagaattatgcagtgctgccataaccatgagtgataacactgcggccaacttacttctgacaacgatcggaggaccgaaggagctaaccgcttttttgcacaacatgggggatcatgtaactcgccttgatcgttgggaaccggagctgaatgaagccataccaaacgacgagcgtgacaccacgatgcctgtagcaatggcaacaacgttgcgcaaactattaactggcgaactacttactctagcttcccggcaacaattaatagactggatggaggcggataaagttgcaggaccacttctgcgctcggcccttccggctggctggtttattgctgataaatctggagccggtgagcgtgggtctcgcggtatcattgcagcactggggccagatggtaagccctcccgtatcgtagttatctacacgacggggagtcaggcaactatggatgaacgaaatagacagatcgctgagataggtgcctcactgattaagcattggtaactgtcagaccaagtttactcatatatactttagattgatttaaaacttcatttttaatttaaaaggatctaggtgaagatcctttttgataatctcatgaccaaaatcccttaacgtgagttttcgttccactgagcgtcagaccccgtagaaaagatcaaaggatcttcttgagatcctttttttctgcgcgtaatctgctgcttgcaaacaaaaaaaccaccgctaccagcggtggtttgtttgccggatcaagagctaccaactctttttccgaaggtaactggcttcagcagagcgcagataccaaatactgtccttctagtgtagccgtagttaggccaccacttcaagaactctgtagcaccgcgtacatacctcgctctgctaatcctgttaccagtggctgctgccagtggcgataagtcgtgtcttaccgggttggactcaagacgatagttaccggataaggcgcagcggtcgggctgaacggggggttcgtgcacacagcccagcttggagcgaacgacctacaccgaactgagatacctacagcgtgagctatgagaaagcgccacgcttcccgaagggagaaaggcggacaggtatccggtaagcggcagggtcggaacaggagagcgcacgagggagcttccagggggaaacgcctggtatctttatagtcctgtcgggtttcgccacctctgacttgagcgtcgatttttgtgatgctcgtcaggggggcggagcctatggaaaaacgccagcaacgcggcctttttacggttcctggccttttgctggccttttgctcacatgttctttcctgcgttatcccctgattctgtggataaccgtattaccgggtttgagtgagctgataccgctcgccgcagccgaacgaccgagcgcagcgagtcagtgagcgaccaagcggaagagc

SEQ ID NO: 7 - DNA, 792 bp, Artificial Sequence
  Synthetic Promoter
aagcttgcatgtctaagctagacccttcagattaaaaataactgaggtaagggcctgggtaggggaggtggtgtgagacgctcctgtctctcctctatctgcccatcggccctttggggaggaggaatgtgcccaaggactaaaaaaaggccatggagccagaggggcgagggcaacagacctttcatgggcaaaccttggggccctgctgtctagcatgccccactacgggtctaggctgcccatgtaaggaggcaaggcctggggacacccgagatgcctggttataattaacccagacatgtggctgcccccccccccccaacacctgctgcctctaaaaataaccctgtccctggtggatcccctgcatgcgaagatcttcgaacaaggctgtgggggactgagggcaggctgtaacaggcttgggggccagggcttatacgtgcctgggactcccaaagtattactgttccatgttcccggcgaagggccagctgtcccccgccagctagactcagcacttagtttaggaaccagtgagcaagtcagcccttggggcagcccatacaaggccatggggctgggcaagctgcacgcctgggtccggggtgggcacggtgcccgggcaacgagctgaaagctcatctgctctcaggggcccctccctggggacagcccctcctggctagtcacaccctgtaggctcctctatataacccaggggcacaggggctgccctcattctaccaccacctccacagcacagacagacactcaggagcagccagc

SEQ ID NO: 8 - DNA, 8629 bp, Adeno-associated virus
gcgcgctcgctcgctcactgaggccgcccgggcaaagcccgggcgtcgggcgacctttggtcgcccggcctcagtgagcgagcgagcgcgcagagagggagtggccaactccatcactaggggttccttgtagttaatgattaacccgccatgctacttatctacgtagccatgctctagagtttaaacaagcttgcatgtctaagctagacccttcagattaaaaataactgaggtaagggcctgggtaggggaggtggtgtgagacgctcctgtctctcctctatctgcccatcggccctttggggaggaggaatgtgcccaaggactaaaaaaaggccatggagccagaggggcgagggcaacagacctttcatgggcaaaccttggggccctgctgtctagcatgccccactacgggtctaggctgcccatgtaaggaggcaaggcctggggacacccgagatgcctggttataattaacccagacatgtggctgcccccccccccccaacacctgctgcctctaaaaataaccctgtccctggtggatcccctgcatgcgaagatcttcgaacaaggctgtgggggactgagggcaggctgtaacaggcttgggggccagggcttatacgtgcctgggactcccaaagtattactgttccatgttcccggcgaagggccagctgtcccccgccagctagactcagcacttagtttaggaaccagtgagcaagtcagcccttggggcagcccatacaaggccatggggctgggcaagctgcacgcctgggtccggggtgggcacggtgcccgggcaacgagctgaaagctcatctgctctcaggggcccctccctggggacagcccctcctggctagtcacaccctgtaggctcctctatataacccaggggcacaggggctgccctcattctaccaccacctccacagcacagacagacactcaggagcagccagcggcgcgcccaggtaagtttagtctttttgtcttttatttcaggtcccggatccggtggtggtgcaaatcaaagaactgctcctcagtggatgttgcctttacttctaggcctgtacggaagtgttacttctgctctaaaagctgcggaattgtacccgcggccgccaccatgctgtggtgggaggaggtggaggattgttatgaaagggaggacgtgcagaagaagacttttaccaagtgggtgaacgctcagttcagcaaatttgggaagcagcacatcgagaatctgttttccgacctgcaggatgggagacggctgctggatctgctggaaggactgactggccagaagctgcccaaagagaaggggagcactagggtgcacgccctgaacaacgtgaacaaagctctgagagtgctgcagaacaacaacgtggatctggtgaatattggcagtactgatatcgtggacgggaaccacaaactgacactgggcctgatctggaacattattctgcactggcaggtgaaaaatgtgatgaagaacatcatggccgggctgcagcagaccaattccgagaagatcctgctgtcttgggtgcggcagagcacccgcaactatccccaggtgaacgtgattaacttcactacatcctggagcgacgggctggccctgaatgctctgattcacagccacaggcctgatctgttcgactggaatagcgtggtgtgccagcagtctgccacacagcgcctggaacatgccttcaatatcgctcggtaccagctggggatcgaaaaactgctggacccagaggatgtggacactacatacccagataaaaagtctattctgatgtacattactagcctgttccaggtgctgccacagcaggtgtctattgaagccattcaggaggtggaaatgctgccccgcccccccaaagtgactaaagaggagcattttcagctgcatcatcagatgcattacagccagcagattaccgtgagcctggctcagggatatgagcgcaccagtagtccaaaaccacggttcaagtcctacgcttatacccaggctgcctacgtgacaactagcgaccctactagatccccctttccatcccagcacctggaggccccagaggacaagagctttgggtccagcctgatggaaagcgaggtgaatctggatcggtaccagacagccctggaggaggtgctgagctggctgctgagtgctgaagacacactgcaggcccagggcgaaatttccaatgacgtggaagtggtgaaggatcagttccacacacacgagggctatatgatggacctgacagctcaccaggggcgcgtgggcaatatcctgcagctgggctctaaactgatcggcaccgggaaactgagtgaggacgaggaaacagaagtgcaggagcagatgaacctgctgaacagccgctgggagtgtctgagagtggctagtatggagaagcagtccaacctgcaccgggtgctgatggacctgcagaaccagaaactgaaagagctgaacgactggctgacaaagactgaggaacgcacaaggaagatggaggaggagccactgggacccgacctggaggatctgaagagacaggtgcagcagcataaggtgctgcaggaggatctggaacaggagcaggtgcgggtgaactccctgacacatatggtggtggtggtggacgaatctagtggagatcacgccaccgccgccctggaggaacagctgaaggtgctgggggaccggtgggccaacatttgccggtggaccgaggacaggtgggtgctgctgcaggacatcctgctgaaatggcagaggctgaccgaggagcagtgtctgtttagtgcttggctgagcgagaaagaggacgccgtgaacaagatccacacaaccggctttaaggatcagaacgaaatgctgtctagcctgcagaaactggctgtgctgaaggccgatctggagaaaaagaagcagagcatgggcaaactgtatagcctgaaacaggacctgctgagcaccctgaagaacaagagcgtgacccagaagacagaagcctggctggataactttgcccgctgctgggacaacctggtgcagaaactggagaaaagtacagctcagatctctcaggctgtgaccacaacccagcctagcctgacccagacaaccgtgatggaaaccgtgaccaccgtgacaacccgcgaacagatcctggtgaaacatgcccaggaagagctgccacctccacctccccagaagaagagaaccctggagcggctgcaggagctgcaggaagccactgacgaactggacctgaagctgaggcaggccgaagtgattaaggggtcttggcagcctgtgggcgatctgctgattgattccctgcaggaccacctggaaaaggtgaaggctctgagaggcgaaattgctccactgaaggagaacgtgagtcatgtgaacgatctggctagacagctgacaacactgggcatccagctgagcccatacaatctgagcacactggaggacctgaataccaggtggaagctgctgcaggtggctgtggaagaccgggtgcggcagctgcatgaggcccatcgcgacttcggaccagccagccagcactttctgagcacatccgtgcaggggccctgggagagggccatttctcccaacaaggtgccctactatattaatcacgagacccagaccacttgttgggaccatcccaagatgacagaactgtaccagtccctggccgatctgaacaacgtgaggtttagcgcttacagaaccgctatgaagctgagacggctgcagaaggccctgtgcctggatctgctgtccctgtccgccgcctgcgatgccctggatcagcataatctgaagcagaacgatcagccaatggatatcctgcagatcatcaactgcctgaccactatctacgacaggctggagcaggagcacaacaacctggtgaacgtgcctctgtgcgtggatatgtgcctgaactggctgctgaacgtgtatgacactgggcgcaccggccggatcagagtgctgagttttaaaactgggattatctccctgtgtaaggcccacctggaggacaagtacaggtacctgttcaagcaggtggctagtagcactggattttgtgaccagcgccgcctgggactgctgctgcatgatagtatccagattcctagacagctgggagaggtggctagtttcggaggatctaacatcgaacccagcgtgcgcagctgtttccagtttgccaataacaaacctgaaatcgaggctgctctgttcctggattggatgcgcctggaaccacagagcatggtgtggctgcctgtgctgcacagagtggctgccgccgaaactgccaagcaccaggctaaatgcaacatctgcaaggaatgtcccattatcggctttcgctacaggagtctgaaacattttaactacgatatttgccagagctgcttcttttccggaagagtggccaaaggacacaagatgcactaccctatggtggaatattgcaccccaactacatctggcgaagatgtgcgcgattttgccaaggtgctgaagaataagtttcggactaagaggtacttcgccaagcacccccgcatggggtatctgccagtgcagacagtgctggaaggagacaatatggagaccgatacaatgtgagcggccgcaataaaagatctttattttcattagatctgtgtgttggttttttgtgtgtctagagtcgaccagagcatggctacgtagataagtagcatggcgggttaatcattaactacaaggaacccctagtgatggagttggccactccctctctgcgcgctcgctcgctcactgaggccgggcgaccaaaggtcgcccgacgcccgggctttgcccgggcggcctcagtgagcgagcgagcgcgcagctgcattaatgaatcggccaacgcgcggggagaggcggtttgcgtattgggcgctcttccgcttcctcgctcactgactcgctgcgctcggtcgttcggctgcggcgagcggtatcagctcactcaaaggcggtaatacggttatccacagaatcaggggataacgcaggaaagaacatgtgagcaaaaggccagcaaaaggccaggaaccgtaaaaaggccgcgttgctggcgtttttccataggctccgcccccctgacgagcatcacaaaaatcgacgctcaagtcagaggtggcgaaacccgacaggactataaagataccaggcgtttccccctggaagctccctcgtgcgctctcctgttccgaccctgccgcttaccggatacctgtccgcctttctcccttcgggaagcgtggcgctttctcatagctcacgctgtaggtatctcagttcggtgtaggtcgttcgctccaagctgggctgtgtgcacgaaccccccgttcagcccgaccgctgcgccttatccggtaactatcgtcttgagtccaacccggtaagacacgacttatcgccactggcagcagccactggtaacaggattagcagagcgaggtatgtaggcggtgctacagagttcttgaagtggtggcctaactacggctacactagaagaacagtatttggtatctgcgctctgctgaagccagttaccttcggaaaaagagttggtagctcttgatccggcaaacaaaccaccgctggtagcggtggtttttttgtttgcaagcagcagattacgcgcagaaaaaaaggatctcaagaagatcctttgatcttttctacggggtctgacgctcagtggaacgaaaactcacgttaagggattttggtcatgagattatcaaaaaggatcttcacctagatccttttaaattaaaaatgaagttttaaatcaatctaaagtatatatgagtaaaaatattccggaattgccagctggggcgccctctggtaaggttgggaagccctgcaaagtaaactggatggctttcttgccgccaaggatctgatggcgcaggggatcaagatctgatcaagagacaggatgaggatcgtttcgcatgattgaacaagatggattgcacgcaggttctccggccgcttgggtggagaggctattcggctatgactgggcacaacagacaatcggctgctctgatgccgccgtgttccggctgtcagcgcaggggcgcccggttctttttgtcaagaccgacctgtccggtgccctgaatgaactgcaggacgaggcagcgcggctatcgtggctggccacgacgggcgttccttgcgcagctgtgctcgacgttgtcactgaagcgggaagggactggctgctattgggcgaagtgccggggcaggatctcctgtcatcccaccttgctcctgccgagaaagtatccatcatggctgatgcaatgcggcggctgcatacgcttgatccggctacctgcccattcgaccaccaagcgaaacatcgcatcgagcgagcacgtactcggatggaagccggtcttgtcgatcaggatgatctggacgaagagcatcaggggctcgcgccagccgaactgttcgccaggctcaaggcgcgcatgcccgacggcgaggatctcgtcgtgacccatggcgatgcctgcttgccgaatatcatggtggaaaatggccgcttttctggattcatcgactgtggccggctgggtgtggcggaccgctatcaggacatagcgttggctacccgtgatattgctgaagagcttggcggcgaatgggctgaccgcttcctcgtgctttacggtatcgccgctcccgattcgcagcgcatcgccttctatcgccttcttgacgagttcttctgaaccggtaatattattgaagcatttatcagggttattgtctcatgagcggatacatatttgaatgtatttagaaaaataaacaaataggggttccgcgcacatttccccgaaaagtgccacctgacgtctaagaaaccattattatcatgacattaacctataaaaataggcgtatcacgaggccctttcgtctcgcgcgtttcggtgatgacggtgaaaacctctgacacatgcagctcccggagacggtcacagcttgtctgtaagcggatgccgggagcagacaagcccgtcagggcgcgtcagcgggtgttggcgggtgtcggggctggcttaactatgcggcatcagagcagattgtactgagagtgcaccatatgcggtgtgaaataccgcacagatgcgtaaggagaaaataccgcatcaggcgattccaacatccaataaatcatacaggcaaggcaaagaattagcaaaattaagcaataaagcctcagagcataaagctaaatcggttgtaccaaaaacattatgaccctgtaatacttttgcgggagaagcctttatttcaacgcaaggataaaaatttttagaaccctcatatattttaaatgcaatgcctgagtaatgtgtaggtaaagattcaaacgggtgagaaaggccggagacagtcaaatcaccatcaatatgatattcaaccgttctagctgataaattcatgccggagagggtagctatttttgagaggtctctacaaaggctatcaggtcattgcctgagagtctggagcaaacaagagaatcgatgaacggtaatcgtaaaactagcatgtcaatcatatgtaccccggttgataatcagaaaagccccaaaaacaggaagattgtataagcaaatatttaaattgtaagcgttaatattttgttaaaattcgcgttaaatttttgttaaatcagctcattttttaaccaataggccgaaatcggcaaaatcccttataaatcaaaagaatagaccgagatagggttgagtgttgttccagtttggaacaagagtccactattaaagaacgtggactccaacgtcaaagggcgaaaaaccgtctatcagggcgatggcccactacgtgaaccatcaccctaatcaagttttttggggtcgaggtgccgtaaagcactaaatcggaaccctaaagggagcccccgatttagagcttgacggggaaagccggcgaacgtggcgagaaaggaagggaagaaagcgaaaggagcgggcgctagggcgctggcaagtgtagcggtcacgctgcgcgtaaccaccacacccgccgcgcttaatgcgccgctacagggcgcgtactatggttgctttgacgagcacgtataacgtgctttcctcgttagaatcagagcgggagctaaacaggaggccgattaaagggattttagacaggaacggtacgccagaatcctgagaagtgtttttataatcagtgaggccaccgagtaaaagagtctgtccatcacgcaaattaaccgttgtcgcaatacttctttgattagtaataacatcacttgcctgagtagaagaactcaaactatcggccttgctggtaatatccagaacaatattaccgccagccattgcaacggaatcgccattcgccattcaggctgcgcaactgttgggaagggcgatcggtgcgggcctcttcgctattacgccagct

SEQ ID NO: 9 - DNA, 4977 bp, Adeno-associated virus
gcgcgctcgctcgctcactgaggccgcccgggcaaagcccgggcgtcgggcgacctttggtcgcccggcctcagtgagcgagcgagcgcgcagagagggagtggccaactccatcactaggggttccttgtagttaatgattaacccgccatgctacttatctacgtagccatgctctagagtttaaacaagcttgcatgtctaagctagacccttcagattaaaaataactgaggtaagggcctgggtaggggaggtggtgtgagacgctcctgtctctcctctatctgcccatcggccctttggggaggaggaatgtgcccaaggactaaaaaaaggccatggagccagaggggcgagggcaacagacctttcatgggcaaaccttggggccctgctgtctagcatgccccactacgggtctaggctgcccatgtaaggaggcaaggcctggggacacccgagatgcctggttataattaacccagacatgtggctgcccccccccccccaacacctgctgcctctaaaaataaccctgtccctggtggatcccctgcatgcgaagatcttcgaacaaggctgtgggggactgagggcaggctgtaacaggcttgggggccagggcttatacgtgcctgggactcccaaagtattactgttccatgttcccggcgaagggccagctgtcccccgccagctagactcagcacttagtttaggaaccagtgagcaagtcagcccttggggcagcccatacaaggccatggggctgggcaagctgcacgcctgggtccggggtgggcacggtgcccgggcaacgagctgaaagctcatctgctctcaggggcccctccctggggacagcccctcctggctagtcacaccctgtaggctcctctatataacccaggggcacaggggctgccctcattctaccaccacctccacagcacagacagacactcaggagcagccagcggcgcgcccaggtaagtttagtctttttgtcttttatttcaggtcccggatccggtggtggtgcaaatcaaagaactgctcctcagtggatgttgcctttacttctaggcctgtacggaagtgttacttctgctctaaaagctgcggaattgtacccgcggccgccaccatgctgtggtgggaggaggtggaggattgttatgaaagggaggacgtgcagaagaagacttttaccaagtgggtgaacgctcagttcagcaaatttgggaagcagcacatcgagaatctgttttccgacctgcaggatgggagacggctgctggatctgctggaaggactgactggccagaagctgcccaaagagaaggggagcactagggtgcacgccctgaacaacgtgaacaaagctctgagagtgctgcagaacaacaacgtggatctggtgaatattggcagtactgatatcgtggacgggaaccacaaactgacactgggcctgatctggaacattattctgcactggcaggtgaaaaatgtgatgaagaacatcatggccgggctgcagcagaccaattccgagaagatcctgctgtcttgggtgcggcagagcacccgcaactatccccaggtgaacgtgattaacttcactacatcctggagcgacgggctggccctgaatgctctgattcacagccacaggcctgatctgttcgactggaatagcgtggtgtgccagcagtctgccacacagcgcctggaacatgccttcaatatcgctcggtaccagctggggatcgaaaaactgctggacccagaggatgtggacactacatacccagataaaaagtctattctgatgtacattactagcctgttccaggtgctgccacagcaggtgtctattgaagccattcaggaggtggaaatgctgccccgcccccccaaagtgactaaagaggagcattttcagctgcatcatcagatgcattacagccagcagattaccgtgagcctggctcagggatatgagcgcaccagtagtccaaaaccacggttcaagtcctacgcttatacccaggctgcctacgtgacaactagcgaccctactagatccccctttccatcccagcacctggaggccccagaggacaagagctttgggtccagcctgatggaaagcgaggtgaatctggatcggtaccagacagccctggaggaggtgctgagctggctgctgagtgctgaagacacactgcaggcccagggcgaaatttccaatgacgtggaagtggtgaaggatcagttccacacacacgagggctatatgatggacctgacagctcaccaggggcgcgtgggcaatatcctgcagctgggctctaaactgatcggcaccgggaaactgagtgaggacgaggaaacagaagtgcaggagcagatgaacctgctgaacagccgctgggagtgtctgagagtggctagtatggagaagcagtccaacctgcaccgggtgctgatggacctgcagaaccagaaactgaaagagctgaacgactggctgacaaagactgaggaacgcacaaggaagatggaggaggagccactgggacccgacctggaggatctgaagagacaggtgcagcagcataaggtgctgcaggaggatctggaacaggagcaggtgcgggtgaactccctgacacatatggtggtggtggtggacgaatctagtggagatcacgccaccgccgccctggaggaacagctgaaggtgctgggggaccggtgggccaacatttgccggtggaccgaggacaggtgggtgctgctgcaggacatcctgctgaaatggcagaggctgaccgaggagcagtgtctgtttagtgcttggctgagcgagaaagaggacgccgtgaacaagatccacacaaccggctttaaggatcagaacgaaatgctgtctagcctgcagaaactggctgtgctgaaggccgatctggagaaaaagaagcagagcatgggcaaactgtatagcctgaaacaggacctgctgagcaccctgaagaacaagagcgtgacccagaagacagaagcctggctggataactttgcccgctgctgggacaacctggtgcagaaactggagaaaagtacagctcagatctctcaggctgtgaccacaacccagcctagcctgacccagacaaccgtgatggaaaccgtgaccaccgtgacaacccgcgaacagatcctggtgaaacatgcccaggaagagctgccacctccacctccccagaagaagagaaccctggagcggctgcaggagctgcaggaagccactgacgaactggacctgaagctgaggcaggccgaagtgattaaggggtcttggcagcctgtgggcgatctgctgattgattccctgcaggaccacctggaaaaggtgaaggctctgagaggcgaaattgctccactgaaggagaacgtgagtcatgtgaacgatctggctagacagctgacaacactgggcatccagctgagcccatacaatctgagcacactggaggacctgaataccaggtggaagctgctgcaggtggctgtggaagaccgggtgcggcagctgcatgaggcccatcgcgacttcggaccagccagccagcactttctgagcacatccgtgcaggggccctgggagagggccatttctcccaacaaggtgccctactatattaatcacgagacccagaccacttgttgggaccatcccaagatgacagaactgtaccagtccctggccgatctgaacaacgtgaggtttagcgcttacagaaccgctatgaagctgagacggctgcagaaggccctgtgcctggatctgctgtccctgtccgccgcctgcgatgccctggatcagcataatctgaagcagaacgatcagccaatggatatcctgcagatcatcaactgcctgaccactatctacgacaggctggagcaggagcacaacaacctggtgaacgtgcctctgtgcgtggatatgtgcctgaactggctgctgaacgtgtatgacactgggcgcaccggccggatcagagtgctgagttttaaaactgggattatctccctgtgtaaggcccacctggaggacaagtacaggtacctgttcaagcaggtggctagtagcactggattttgtgaccagcgccgcctgggactgctgctgcatgatagtatccagattcctagacagctgggagaggtggctagtttcggaggatctaacatcgaacccagcgtgcgcagctgtttccagtttgccaataacaaacctgaaatcgaggctgctctgttcctggattggatgcgcctggaaccacagagcatggtgtggctgcctgtgctgcacagagtggctgccgccgaaactgccaagcaccaggctaaatgcaacatctgcaaggaatgtcccattatcggctttcgctacaggagtctgaaacattttaactacgatatttgccagagctgcttcttttccggaagagtggccaaaggacacaagatgcactaccctatggtggaatattgcaccccaactacatctggcgaagatgtgcgcgattttgccaaggtgctgaagaataagtttcggactaagaggtacttcgccaagcacccccgcatggggtatctgccagtgcagacagtgctggaaggagacaatatggagaccgatacaatgtgagcggccgcaataaaagatctttattttcattagatctgtgtgttggttttttgtgtgtctagagtcgaccagagcatggctacgtagataagtagcatggcgggttaatcattaactacaaggaacccctagtgatggagttggccactccctctctgcgcgctcgctcgctcactgaggccgggcgaccaaaggtcgcccgacgcccgggctttgcccgggcggcctcagtgagcgagcgagcgcgc